European Patent Application EP 4 782 545 A1, published July 29, 2026. Title: 一种蛋白复合物的制备纯化及应用. Applicant: 北京朝赛蕴生物科技有限公司. Application WO. The sequence listing filed with the application follows.

SEQUENCE LISTING (69 sequences)

SEQ ID NO: 1 - DNA, 450 bp, synthetic construct
  source 1..450: mol_type = other DNA
atgtctacaagcacatctcagattgctgttgaataccctattccttcttatcgtttcgttgtttccgtcggagatgaacatattccatttaatagtgtttcagggctggatattaattatgaaaccattgaataccgtgatggcgtgggtagttggtttaaaatgccgggtcagcgtcagccgattaatattaccctgcgtaaaggtgtttttccgggcaaaactgaattatttgactggattaattctatccaacttaatcaggttgagaaaaaagatatttccattagtttaaccaatgacgcaggcactgaattattaatgacctggaatgttgctaatgctttccctacctcattgacgtctccttcctttgatgccaccagcaatgatattgccgttcaggaaattaccctgacagccgatcgcgtcaccatgcaggctgtttga

SEQ ID NO: 2 - DNA, 1068 bp, synthetic construct
  source 1..1068: mol_type = other DNA
atgacaaccgttaccagttatcctggcgtttatattgaagaattaaatagcctggcattatccgtatcaaatagtgccaccgccgttcctgtttttgcagtgaacaaagaaaacaaacagattaatgaagagactgcacaccgaattaattcctggatggattatcttaatctggtaggcaactttgacaatgaggataaattgtcagtttctctgcgggcttattttaccaatggcgggggttattgttatctcatcaaaaccccaaatttagaaaaacttattccaaccttagatgatgtcactttgctggttgcggcaggtgaagatattaaaacagccgcggcaactttatgtcagccgggaaaagggttatttgccatttttgatggccctgaagaagcgttgaccatcgcgaatgcagaaacagtcaagaacaaatatgacgccaccgcgttcgccgcagtttactacccgtggctgaaaacggattgggcaaaaatcaccattccaccgagtgcggttatggcaggcgtttacgcctccgtcgatctctcccgtggcgtgtggaaagctcccgccaatatcgcattgaaaggcggactggaacctgcatttttgatcacggatgaagttcagagtgcatataactccggtcgtgccatcaatatgattcggaatttcagcaataccggtgccaccgtttggggagcaaggacgctggaagataatgacaactggcgctatgtccctgtgcgtcgcttattcaataccgtcgagcgggatgttaagcgcgctatgagctttgccatgtttgaacctaacagccaaccaacgtgggaacgtgtcagggcggcaatcagcaattaccttcatagcctgtggcaacaagggggattggctggcagcaaagaagaagatgcctatttcgtgcagattggcaaaggaattacgatgacgccagaccaaattaatcagggacaaatgatagtaaaaatcggcctggcggccgttcgaccggcagaatttatcatcctccagtttacgcaagatgtagaacagcgttaa

SEQ ID NO: 3 - DNA, 1437 bp, synthetic construct
  source 1..1437: mol_type = other DNA
atgccagctaatctaaaaacgcccggcgtttatattgaagaagatgcttcccttgcattatcggtcagcaacagtcccactgccgtgcctgtttttattggtaagttcaccccaaaaactgcggagccaacccaaacctgtattcgtatcagcaattggcttgaatttacttcctctttttctttggcaccagtgacagaaattgtcatccgctctagtcttgaagcctcttctgatggcgcaacaaaaaaagaacaggccaaaaaagaaaaagtcgaaaataaagagactgcaacccaagaaactcccaaagttcaaactctctcggcagccgaagaagaacccaaaaaatggattcacaatattgagagagtcaatctatctcaagccgtagaagccttgaagctctattttcaaaatggaggcggggcttgttatatctacccattaaacaatattaatggcgagtcggctctggaccccattcctaaggtgatagaacaaaaaggggatatcactctgttggtttgtccagaagaagatcagggttataaaaacagagtctacagtgcagtcagccccctattgaatagtgataacaaaaaagtgggctatttcctgattgcagatagccttgatggtaaatcggtgtctggcatggcaaatagcaccaagatcgccgcctattatcctcagttggaaacaaacctgaaattctccaccttgcccgacgatcagaacattgttatcagtggttatgagaacgcatcaggcaaggacaagctgaaaactctggataaacttagggaaacagataaagcgctggcacaagaaattgatatcagattgcaagaaatacaacaagataatctcaccctttcacccagtgctgccatcgcaggaatttattgccaaactgatagccagcgtggcgtctggaaagctcccgccaacgttgcactcagcggaatcaaaggtctgactgataaagtcgatgacgaacggcaaggcaccatgaatgagaatggcatcaatgtcatccgttcatttaccggccgtggcttgatggtttggggggcgcgtacttatgctcagaacggtgagatcaactggcgttacattcctgtccgtcgcctgttcaattccgttgaacgtgatatccgtcaggcactgcgtgccgtgttatttgaaaccaataatcaaccgacatggatgcgcgccaaggctgccgttgaccaatatctttatgccctctggcaaaaaaatgccctgatggggaacagcccggaagaggcttattttgtccatatcggtcaggatatcaccatgtctgatgcagatatcaaacaaggcaaaatgatcatgaaagtaggtctggccgcagtgcgaccggctgaatttatcgtcctgcaatttacgcaggatgtcgctcagtaa

SEQ ID NO: 4 - DNA, 1209 bp, synthetic construct
  source 1..1209: mol_type = other DNA
atggaaagaattcaaccgggcgtgaccttgacagaaagtataattaccacaggccagcaagagatacccagcgcagtgccggtatttattggctataccgtccgcaatcaacaacaagcaaaaaccgcagttcgtatcgacaatctggcggaatatacccagcgatttggcgacgatcatctgatggcattggcggtaaggcactatttcgataatggcggacaacgggcttttgttttgccactgtcaggaaatatgccctcagcaaacatgacccaagcggaagccgaagcactgatggcggcattaagctctgacatggtgcaagaagccattggtggggaaacgcagatcaccctgattttggcaccggatatcgcccgactgaatgacaatgtgactgatgagcaacaaactttagtcaatttgtggtcacagggttggagtacactgctgcaactaagccagatccgcacgaatctctttgtgctgctggatgcgccggatgaggttgaacaggcacggcaatgtctggaaggactctcgtcagagtatcgccaatggggagccgcttattggcctcgtctggaaaccacttatcaggctacatccagttccaaaaatattatgctctcccccactgccgctatcgcagcacttatccaacacacggatagcgaagttggtgtatggaaagcgccagccaatattgccctgtctcaggttatccggccggttaagtcgtatcttcaagggagtgtactgtttgacaccaatggcacttcgctcaatgtgatccgcactttccccggcaaaggcatacgcgtatggggatgccgcacactggaaaacacagataacacgcagtggcgttacctacaaacacgacgtctggtttcttatgtcaccgtacatttggcgcaattagcccgtatgtacatctttgaacctaataacgaactgacgtggatgaaatgcaagggacaaagttacaactggctacggcaactgtggttacagggtggcttgtacggctcacgggaagatgaggcatttactgtgctgttaggcgtcaatgaaacgatgaccgaagaggatattcgtgccgggaaaatgataatgaaagtcgccttagccgtattgtctcccgcggaatttatcgagatcagtttggtatttgatacccaaacgggcgcgcttttgtcttaa

SEQ ID NO: 5 - DNA, 459 bp, synthetic construct
  source 1..459: mol_type = other DNA
atgaacgattattacacccccgtggtatcccaccgttttatggcgagctttatttttaatggcattcctgatccactggatatccgttttcaacgtatttccggcctgaaccgggaacttcaggtcacccagcacagccaaggcggtgaaaacgcccgcaataactatctggctgaaaaaatccaacacggcacattaacgctggagcgcggtgtgatgacggtttctcctttgacctggatgtttgaccgtgtattgcgtggagaaaatatcgcctatgcggatgtggtgattatgctgttaaacgaaaattcgctgcccttgtccagttggacgctgagcaatgccttaccggtacgctggcagaccagcgattttgacgcgaacagtaatgccattctggtgaatacccttgaattgcgttatcaggatatgtgctggctgggagtcaaagtatga

SEQ ID NO: 6 - DNA, 198 bp, synthetic construct
  source 1..198: mol_type = other DNA
atgaccgtcgaaatcagagaattaattattcaggcaaaagtggtttcatcatcaccaatactcccaacacaagcaactgaatcacatcaacaaagccattctttgattcaggaaagtctggatgaggcagctttagttgaaaaaattaaacgcgaagtgctggctgcattacgcgatgaggaaggatggcgcccatga

SEQ ID NO: 7 - DNA, 687 bp, synthetic construct
  source 1..687: mol_type = other DNA
atgagtttaattgaacgtggtttagcgaagctgacgattaacgcttataaagacagggaaggaaaaatacgggctggcaccattcaggccatgtataaccctgattccctgcaactggattaccaaacggattaccaacaatcccaggcaattaatagcgaaaagcagagcagcatttatgtacaggccaagcctgccgggttatcccttgagctgatttttgacgccacaatgccgggcaacaaaacccctgttgaagctcagttaatgcagctcaagcagttgtgcagcgtggatgccaccagtaacgaaacgcggttcctgcaaatcaaatggggaaaaatgcgttgggaaaaccgcggctattttgctggcagggcgaaaggtttgtctgtgaattacaccttgtttgatcgtgatgccacgccattgcgggcgcgggtcatcctgacattggtggcggatgaaagtctggtcttacaggagacagagcaaaacctgaaatcgccggcgaaaattgccttacgggtacaggatggtgtttcgctggccctgatggcggcaagcaccgcatcaacgctgtctggtggtgttgattacctgacgctggcctggcaaaacggtctggataatcttaacggatttgtaccgggtgagatattgcaggccaccagaggagatgcctga

SEQ ID NO: 8 - DNA, 1617 bp, synthetic construct
  source 1..1617: mol_type = other DNA
atgagccatcaactgaaaatcattgccgatggcaaggcactgtctttgctggccgccgttgatgtcgatacttactgccgcgttaacagcatcccttccgcaacgctgaaactcagcctgccggacagccctctttcctctttcagccaaacggatgtacaggcagaactggcccattgtcaggcagggaaaaccctgcgtctggaattgactgacagcggcagaaaatcagtgctgtttaacggcctgattacccgtaactctttgaagataaaaaacaagcaattattgcttactttggttgtccgacatcggttgcaactgatggcagatactcagcactcacaactgtttaaggccagtaatgaaaaaaccattctgaacaccttattgaatcaggcgggtatcaaggctcgttttgagcggatagacgcactggatcaaaaacatgaacagatggtgcaatttcgctgttcagactggcgttttctgttgtgccgactatcggcaaccggcgtatggctgttacccacgacagaaggtgctcagcttgtccagcctaacaccctgaaatccaacccaacccataccctgaaaagccggggagatgagaaaaaagatatcatcgtcaaggatgccaactggcagtttgataaccatcttaaccctgcttcgctggaagtcagcggctgggatatcagtaaacagcaagaattatcaggtggtcgccacggcagtgttgccatgggcaaagccgcactttctcctgacaggctggcgtctttaaataaaacaagctgggacattcgctacagcagcccgttaaccacccaagagagtggctatctggcacagggactgttgttgaatcagcgcatttctggtgttacaggcgaattcctgcttaaaggtgatggacgttatcagttaggggacaacattcaattaacgggatttggttcacagctggatggaacagcaagcattactgcggttcgccatcgttttaaccggcgaattgattgggaaaccactttaagcattggcttaccacaggaatatctgccgatgctacccgatgccaccggactccatattgcgacagtcgcgaagtatcagcaggacaaggcagccctgaaccgcattccgattattctgccggtactgaatcgtccgaatgaattcttgtgggccagattagggaaaccttacgccagccacgaaagtggtttctgtttttacccagaacccggtgacgaagtgattgtcggcttttttgaaaatgatcctcgttatccggtgattctgggggcaatgcacaacccgaaaaataaagcgcctttagaacccacccaggataatcaggaaaaagtcttggtggtgaaaaaaggagaaatccaacaacaaatcatgattaatcgcaaagagaaaactattcaaatgagtgcaggagaaaaccagataatgctccagcaggataaagatatttcgctgtcaacgaaaaaagaattaacactgaaagcgcagaccatgaatgccgaaatggagaaatcactcaatatttctggcaaaaacagtgttgagatcaaaggcagcaaaattaatcttacccaatga

SEQ ID NO: 9 - DNA, 423 bp, synthetic construct
  source 1..423: mol_type = other DNA
atggaaaaccaaatactgacacagctttatggtcgtggctgggcttttcctcccgtcttttcccttgaaaagggggtggaaatggctgaggggacagaagatgtgcgccaaagtttgcatattctgttcagtactgagccgggggaacgcctgatgcgcgaaaattacggctgtggattaaatgattttatgtttgaaaatatccgcaacgaactgtttgctgaaattgaatcccatatccatgacagcgtattacgttatgaatcacgggcagatattaccgatatccaagttcgtcagtcgccaaatagcaaaaataccttgcaagtgcaggtgatgtatcgcctgcggggcagcgatatcaatcagcaaattcaaggaacactggcgctgggtgaaggccagggaatggaggtggtatga

SEQ ID NO: 10 - DNA, 432 bp, synthetic construct
  source 1..432: mol_type = other DNA
atgagtgaacccattgtaactgacggcgacacattacagtttgagccccaatttgagagtcgaaaggtgaacattcccggattgattaaaatcaatggaacaggtcatgcacaggtcaacggcaaaaaagtttgcattttgggagacgagaaacgggttactgtttctgcaacttataccacaacaactcatatgacaccgggaactggcaccattactatcacggcgttagatagcagccagcaagcccttcaatgtaccagtgatgctgctttaattatcaaagggaaaaaatttacggccatatttacgcctcaatcaccagccataaatggtaatgtgaatccacctcaacctgatcctaattacccaagcccttcatcaggcaaaggcagttttatcacccaacaaaactttgccactgtgaattaa

SEQ ID NO: 11 - DNA, 2211 bp, synthetic construct
  source 1..2211: mol_type = other DNA
atggaattaactgagttaaataaaaaattgtcagatttggtgccgatgagcgattttaaattagatagccgaaccagtttgcaattactccaatatattgaggagtacactaaaataattccctttaatcaaaccgataagcattggaatgattttttctttaagaaagatagtacgccagagaaactggccgaattatatcaagggaaaatcgaagccaatgggaatttattacctcatcaagcttttctactagcggtattacgattactggaaacaccaatatccttattgaataccttaccggcggcgcatcgcaatctctattatcgggcgcttttggggctatctccccgtccggctcgacctgatcaagttgccttatctgtagaactgaataccacagtcacagaacaactactcactaaaggcactttatttgaagcagggcaagatgaacacggcaatgccttgcaatatgcgctggataccagtttgctggcaaaccgtggctatattagtgaattgcgctggctccgtaaaaaagaacaacagcaatggatcaccgcgactccctggaattcacaggcacaattatcattgccatctggtggaatacggttattcagtgaaactgatttggataaatcggtactgggcgggatgttgatcacttccaaacatctggcgatggaagaaggagcaagagagataacgattacctttgataaggacatggatagccagaatttggtggcacaaatcagaagtggtaatcaatggctaactttacaagttgagaaaaatacagctgagagaaataaaaaagaagtcataatgatgctggcagataaagagccagcaacccgtgcaccagaggatctggataacctgattttcagtgagccagtactcaggctacagggaaaaaacagccaaccactgcctacagtcaccgcactaaaggtgcaaaaaacaactatagataaagcttcattcaagacatttcacttaaccccctttggttatagccctgaaattgaaccattggaagaaaaccccgcattataccttggtatcactgacgtcaagccgggacaaaccctatcgctgtattggaaattaaaatcgccacagcaacccgaaaacgttttctggtattacctgaataataagaatcaatgggttgcattagatgcgtgggtcaaagatgaaaccaaatatctgtatcaagatggcatctggcaagttgtattgcctgcggatgcttctgcttctgctgaagaaattacccggatgccaacagggcgctattggttaaaggcagtcatggttatccccacacacaaaggttcatggggaaaaactccttggttagacggcttgatctataacgccatgacagcgacattaacgaatgccgatagcatcagcaacagccatttcttgacgccattaccggcagacactattcaacgtcccgttgagcctatcatggaggtggcttcgatcagtcagccttggccgtcgtggaatgggcgtgtaccggaatcctacagcgctttttttgcacggggagctcaacatctgtcccaccgtaaccgcgccttaacctggggcaatatggcgacactgttaaaagagcgttatgtcagcatttttgatgttaagtaccccggccatgatgaactcacgcgagtccccgcactggagaaacagcaactgaccatcattccggctaaccaatacaacgacagcgatgatcctttgcgtccggtgttaaaccctgcccgcctgcaaggaatggccgaatggttacagcaaaaaggctctccatgggctgagattgagatcagcaatcctcaatacattgatgtaaaaatcaattacaacgtgatttttaagccggatgttaacgaagattttggttatcgccagctacgacagcaactcagcgagacatatatgccctggagcgtcgatgagaaacgccccgtcacgctgaataacagcattagttattaccaattactggcaactatccaacagcagccgctggttgagcgggtcacttgtctgacgctgcgtcggtcggaagcggctaaagacagtgatatcaccgcatcagtggaagccaaagataatgaagtgctgattttggtctgggaagcagatgacaagctgcaatgccgaggaaataactatgagtaa

SEQ ID NO: 12 - DNA, 2892 bp, synthetic construct
  source 1..2892: mol_type = other DNA
atgagtaatcaagatgcactatttcacagtgtgaaagacgatattcactttgataccttgctggaacaggctcatcaggtggttgagcaacaggcaggaaaattgtggagcgacacagcggaacacgatcccggtatcacctttctggaaggactcagttacggtgtgtcagatttagcttaccgtcatactcttcctccgacagacttactgacccctgcccctaatgagcagaaacagcaagatggaatttttcccgctgaatttggcccccacaatacactgacttgtgggccaatcaccactgatgattatcggaaggcattacttgatctgcatagcagtgactggacaggagcaaagccagagtcagaacaggacaaaggggattttctgttccgtaacgtgcaactggtacgtgaaccggaaacacaacgctatacctattggtatgatgccaccaaaagggaatatagctttgtcgagcgtaaagatgcgaaaaagtttaccctgcggggaaattattggctttatctggaaccgacccgtcgtactcaggagaatttggataatgctacccaacaattaatcgattttttgactcaaaaccgcaatattggtgaattggtcagtcagagaatctggacaaaaccggttgattttccgctattactggatattgaactggatgacgatgtgcaaaatgtcgctggtatttttgctgccgtctatagcacagcagaacagtatctgatgcctgaggcgcagcgtttcagtaccgaaacactacaagatgcggaaatgcgtaatgatgaaatctttgaaggaccacgattagaacatggctggatccctgaattgccgacagcccgtgattataccaaacggctcaagctcaatcttagccggctggtcaataagctgcttgagattaagggaatacagaatgtaaatcgtcttcgactgaatgaaaattttgataagaccctgattgagccgattaaaggggatagctggtcatggtcaataaaagaaggctactaccctcgtttgtggggtaaagatccgattcatcaattggcacaacatgatggcccactgagggtgatcgccaaaggtgggatcagcgttacggttgatgaaaacagcattcgaaaaagtttatccttatcccatcctcctcttattcagaataaacctgtgctattggcttatggtcggcatcgcgatgtgggtcgctattaccccgtcagcgatacgttgcccgcttgctacaaattacagcagcctttatctgaaagtgaacatgcgcaacgcctgttatcacttcatcaatttatgctgccatttgaacaattgttggcttgcggctgccagcaaattgccatgctgccaaaattgttggcttttaagcgtgagggatatgaagtttggggtgatcaatggccatttaagccgggttctgtcaatgatgatgcccaccaaaattacgcttacgaattaaagaaagtactaaaagagattgcacacgataacgatcacgaattggatattgtcaattatctgctcggatactttggcactcagcgagcaccacgtacctttaccaccaacatcagtgattttcgtgccgtgcaacaaggctatctggctcaacaaccgacattaacttatcaccgagccaatattcggatcgatcaagtttcgtcgctacaaaagcgcattgctgcccgtatggggttagggggtgaattatttaaaccaaagcctgacttgagcaaactgcctttttatctggtagaacatcgggcattgctgccagtcaaacccaacagccagtttgatgaagagcagaagccagattcggtgacagaagaaaggaactatcaaaatgatcaatattacttggtgattaagcaagccggtattgatggaaaactgatacagggacaggtaattgatttagttctctatgaaggagaacagaacgaaaaccgatttaccgtgcgtggtcaaatgatcactaaaaccacaggagatcagttttggctggacgtgagcaacagtactcaactggaatacaatctggaacgggtaatgaccgccgccaaagggaaaaaactcgtctggcaaaatagcccggtatggatggaagatatgaactaccggctggcctatgatagtgatcaatcctcattgcctgaaaaccagcggcgcctgacccgcacagcacaaacccccttcccggccctgattgccgcaggtaatgaaattaccctgacaaaacagttggggggagtgggtttggagcaagaatcttctaatgaatcagaaaaattatatgcaaaagttgtcagctttgatcgcatcaagggaactttgattattgagcgtcagaaacattctacactggcattccctgccgcagaagaagcctggcggcacagttggcatttttcgggtaaggaatatgaaaatacggaccgtttctcatttgtgattagcgtggtggtaaatagtgatttaattaaatcacgtgagctcaaagttgatccatatcaattggaagagtgggttaaggaaactattctcaccgaattccctgcccatatttccatgattattcactggatggatcgggagccatttttaaacttcggcaatacgtatcaacgttggcaaaataatggcgcaccattaggggatgccgcttattcgattctggaaagtttgacgctgggtaaattaccttccgctttcaaaggaattgggtcaatgcgtattgccacaccacatcagagagaggaagttgttggtaagaatggtgaacaatggaataccaatagaataaaacaaaacgaattattctatattccgaaagagaaagaataa

SEQ ID NO: 13 - DNA, 1260 bp, synthetic construct
  source 1..1260: mol_type = other DNA
atgaaagaaattcgttattctgcaaaaatacaagaacaacaaacattatctgacgcaaaaggtgttggacctgatattgataaattaaaagataagtttaaagaaggcagtattcccttacaaaccgatttcaatcaattaattgatattgccgatattgggcgtaaagcgactggacaggctcccaatcaaaatggcccggcaaaaggaatgcgtttgggcgaagatgggcttttacagttaaagttagatgagaaatacgctcatgcaaattacagtccattaagattgcatgatgatgcattggttgtaggagtaggcaatggtttgataaattttaaaaaatcaaatgaaataggtgttaatgatggaaatggtattaggatagatgataataaggttgcagtagaactggctgataataaaggtttggttgttgatagcaatggtatcgccataaaaccaggcaatggggtgaagtttagttcagatggtgcattaacagtaaattcggctgattcaactattaaagttgatggctcaggaataaaagttgctacaggttggggagttaaagttggtggtgaaggtttggatgtaaatgtccgcacggatggtggtattggtaatgattcgtcaggtatttatgttaaaacaggtaatggtattaagttagataatgatcaagttgcagtagaactagctgataataaaggtttagttgttgatagtaatggtatcgccataaaacccggcgatggaatgcaatttagttcagatggtgcattacagttaaaattaaataagaattatgccgatagattttatagccctttaatattgcgtaatgatgtattggctgtaggtataagccatggtttgacaacttatcaaggatcatatgcaataggtgttaatccaggaaatggtcttaggataaatgacgatagtgttgcagtgaaactagctgataataaaggcttggttgttgatagcaatggtatctccataaaaccaggcaatggaattaaggtagatgctgatggtgtggctatcgatcctaatactgtattgccacgtggtatgattatgatgttttctggtaatagcgtaccagaaggttgggctatttgtgatggctataataatacaccagattttctaaatagatctattgagggaaatactaggaatattaaaagtaaaaatggtatagatatgactatacaatatactgcaatatatatcatgaaattataa

SEQ ID NO: 14 - DNA, 1536 bp, synthetic construct
  source 1..1536: mol_type = other DNA
atgatgaccaacactgataaatatggtgttaatcttattaatagaataactatctccattgatatgttatattttaacgatgataacataatggagaactgctcatctatatttaatagaaaactaaaaaatatcatcaataaaaatatcaaaaacctgacattgaatgtaaatgggaagttatctcttgaaagggtaactctggatctgggaaatattgaaattgatttatttgaaagggaaataacaagaagattggaaatagaattaaaaaagaacttaagaaatcattatggttactctcaatgtattttaaataaagagaaaatatatccacaccaatcagaaaaagaaaatagatttttattaataaaagaaatagatcattacttacataagggaaactggttatctgatcacagaaagcatcatattacaaatactgtgcatattaataatgaattatggcaacagattaaccaccagccacaacaatggctacctatgttagccaaacactgcttacagcctgcggggctaagtcgcttaattcaactctgccagccagacgttcttgctatgctttgccagttatttactgaaacaacaacatccgaatttgttaattcgcaagcgcaggtaattacagataaaaaagtgaaaccagaaaaattgagtttggctgcggaatattatctgcaacatcaggtgaaatatccccatgccacacaacaagcacttgcacaacaaactcaaaataagcaaacaccgacaataaatattattcagaataataacagtctattaaaacagacttacaatgaaactgatatgcagatggatacagtactgccatttgcaacataccatcagccaacagctacgcaacagcattatggtcttataaaagaggcggtaaaacaaagtcttccaactttacaaaacagagagcaacataaggaattaccgagatcaacttcaccagcgaaaatatcatccatacaacccagtaatggaattcagactccatcatcacaatccgttttaaccatcagcaatgccggttgcatgattttatggccgttattgcccatatttttccgtacctttgatttactggaaaagaatcaatttatcagccttgaagcacaaagagaggcggtctgtttacttgattggctgatttgggaagaagaggaaatacctgcatggcgattgactctcaataaaatactttgtggattacccatacatgacaacgcgcgatggcgtaccccaaagccagaacaacaaattgccatcaaccaatggctggaaaaaatcatcgaacaacttccagcctggaaaaaaatgggaataaacgatgtgcgacacttatttctgcaacgttccggggaattaagtgagttaaatggaataaaaaacatccatattaaacccgaagtttatgatgcactgataagcgaatgggcgtggccaatgaatatcgcgagctttagctggttgcaacaccctatcaccataacgtggtcataa

SEQ ID NO: 15 - DNA, 2088 bp, synthetic construct
  source 1..2088: mol_type = other DNA
atgaatacagcgcctgttttccctgatttatttcagcaacataatgatcctcatttaatgttcttatatagccaactggaacgcatcgatctcgttctgcaataccatttccattgcatatcaggccagaaaggtgacctccttgatgagttcttgttaagcgaagaagatgtgataaacagactggataaccctctgggaaaacctcattggctcaccgatgattgcctgacaataccgcacaccgtcacgcccgtggcatcccgattaactgacctgattacacattttgaactgactgattttgaaagggatgttttgttgttaggtttactgccccatttcgataaccgctactatcacctgtttgctctggttcagggagaacaacaatctcggctgcccgcttttgcgttggctttggaactgttttgccactcaatgctggaaaaacaggcacagcaggccagttttttacaccaggctcccttggttggctgccaactgttatctattgatagtcgtcagaaaacgttatcctggctccagacaccctttatcacagacagcagcgtatatcattttttacttgggcatcactatattgcacctgctctggaacattgtgttgagtggataacgcccacagaaatcggcaattatccagcaggattaaaacaagcgttgggtaatgtactgttatctgatcatgatgatatccggcccgttatcttactgcggggcatggccgatagtgccagatcccatgtcgttgctaatatgatggcatcagaacaacggcaaacgctgcttgtggatatcgccagcttagctgataacgatgacaactccctgttttgccatataaaagccattttgcgagaaattcgtatgcgtggtgcctgtttattgttacgaaacttttgcttatttgcagaacagaataaacacttgctggatcccctgtcagccttattaaaccaatctgaattaagggttatctgtctggttgaaccacactcaccgttagtatggctgaaaaagatatcgacattactgatcgaaatgcccgctttcacttcggtggaaaaagcaagattattgacggcccatttacccaatcactgtgcaaatgatatagatgcaataaccttaagccaacgttacgcatttaatcctgaaaccctgccattaattttacaagaggcgaaactttaccagcaacagcgagatccttcaggtattttgcagcaatgtgatatccataaggcactcaatttacgcgcccagcaaaattttggtcaattggcacaacgcattacccctaaacgttcattaaaagatttattggtatctgatgatattgctcaacagatacaagaaatactcgcagccattaagtatcgggaacacgtcctggcgggaggttttaaagataagattggttatggtacgggtatcagcgccctgttttatggtgattctggcaccggaaaaactatggcagcagaagtgattgccaattacattggcgttgacttaatcaaagtggatttatctaccgtcgtgaataaatacatcggcgaaacagagaaaaacttatcccgtatcttcgatttggcagaacaggatgccggtgttttattctttgatgaagcggatgcgttatttggtaaacgcagtgaaaccaaagatgcgcaagaccgacatgccaatattgaagtctcttatctactgcaacggctggagaactatccggggttggttattttatccaccaataatcgtagccatttggacaacgcctttaatcgccgttttacctttattacccgctttacttacccggatgaaaccatccgcaagaaaatgtggcaggcaatctggcctgaaaatataaaagtcgcccaggatgtggatttcgataaattagctcaacgaacaagcgtaacaggggcgaatattcgtaatattgctttattgtcttcactgtttgccgcagagaataaccataatgaagtcagtaataaaaatattgaaacagcattatcacgagaattagccaaagtaggccgtttaattttttaa

SEQ ID NO: 16 - DNA, 906 bp, synthetic construct
  source 1..906: mol_type = other DNA
atgttaaaaacgcaaaccattattgatgtcaataacgcaatgaaaactatgctggagaaatatctggataataaaattgcaattcgttttgacttacctgaattagataccgtgcaatctgatgcgatggtgagtgtctttctgtatgatatccacgaagatctacagcttcgttcgacagaatccagagtgtttaatgccacttcagggagattattgccgggttgggtcaatattaaatgtaattacctgattacctattgggaatcggctcaaccagcaaccgattccaacagctcagaatgtctaccggataatcaggcaataaaagtcatgtcacaagtcttgaatgctctgattaataatcgccaattggcaggtattcccggtgcttatactcaggttgtccccccgaaagaaagtttaaacagtttagggaatttttggcaatcactggggaatcgcccccgactttctttaaattactcagtgacaataccgattagcctcaccgataagcaggataaggcgacgccggtaagcaccatttcttctacagtggaacaaattgcatcactcagtcaggaaaagattagccatactttgcgagaattattgattacggaactacagatacaacctgttacagaatcagaaagtgaagagaatatcaggctggcactgagcaaagttgaactattaacaatgaaaaaggctataactccagacaattcagcagaaatttccatatccttgtctgtatcaggtattacccatcagaaatatctacaggatatcaataaaatttttgatcgctggttaaatgacaacaaaattgttactacagtcgataattatggaatcaggattaaggatatagaaaaaaaccatcttttcggcatttaa

SEQ ID NO: 17 - protein, 149 aa, synthetic construct
MSTSTSQIAVEYPIPSYRFVVSVGDEHIPFNSVSGLDINYETIEYRDGVGSWFKMPGQRQPINITLRKGVFPGKTELFDWINSIQLNQVEKKDISISLTNDAGTELLMTWNVANAFPTSLTSPSFDATSNDIAVQEITLTADRVTMQAV

SEQ ID NO: 18 - protein, 355 aa, synthetic construct
MTTVTSYPGVYIEELNSLALSVSNSATAVPVFAVNKENKQINEETAHRINSWMDYLNLVGNFDNEDKLSVSLRAYFTNGGGYCYLIKTPNLEKLIPTLDDVTLLVAAGEDIKTAAATLCQPGKGLFAIFDGPEEALTIANAETVKNKYDATAFAAVYYPWLKTDWAKITIPPSAVMAGVYASVDLSRGVWKAPANIALKGGLEPAFLITDEVQSAYNSGRAINMIRNFSNTGATVWGARTLEDNDNWRYVPVRRLFNTVERDVKRAMSFAMFEPNSQPTWERVRAAISNYLHSLWQQGGLAGSKEEDAYFVQIGKGITMTPDQINQGQMIVKIGLAAVRPAEFIILQFTQDVEQR

SEQ ID NO: 19 - protein, 478 aa, synthetic construct
MPANLKTPGVYIEEDASLALSVSNSPTAVPVFIGKFTPKTAEPTQTCIRISNWLEFTSSFSLAPVTEIVIRSSLEASSDGATKKEQAKKEKVENKETATQETPKVQTLSAAEEEPKKWIHNIERVNLSQAVEALKLYFQNGGGACYIYPLNNINGESALDPIPKVIEQKGDITLLVCPEEDQGYKNRVYSAVSPLLNSDNKKVGYFLIADSLDGKSVSGMANSTKIAAYYPQLETNLKFSTLPDDQNIVISGYENASGKDKLKTLDKLRETDKALAQEIDIRLQEIQQDNLTLSPSAAIAGIYCQTDSQRGVWKAPANVALSGIKGLTDKVDDERQGTMNENGINVIRSFTGRGLMVWGARTYAQNGEINWRYIPVRRLFNSVERDIRQALRAVLFETNNQPTWMRAKAAVDQYLYALWQKNALMGNSPEEAYFVHIGQDITMSDADIKQGKMIMKVGLAAVRPAEFIVLQFTQDVAQ

SEQ ID NO: 20 - protein, 402 aa, synthetic construct
MERIQPGVTLTESIITTGQQEIPSAVPVFIGYTVRNQQQAKTAVRIDNLAEYTQRFGDDHLMALAVRHYFDNGGQRAFVLPLSGNMPSANMTQAEAEALMAALSSDMVQEAIGGETQITLILAPDIARLNDNVTDEQQTLVNLWSQGWSTLLQLSQIRTNLFVLLDAPDEVEQARQCLEGLSSEYRQWGAAYWPRLETTYQATSSSKNIMLSPTAAIAALIQHTDSEVGVWKAPANIALSQVIRPVKSYLQGSVLFDTNGTSLNVIRTFPGKGIRVWGCRTLENTDNTQWRYLQTRRLVSYVTVHLAQLARMYIFEPNNELTWMKCKGQSYNWLRQLWLQGGLYGSREDEAFTVLLGVNETMTEEDIRAGKMIMKVALAVLSPAEFIEISLVFDTQTGALLS

SEQ ID NO: 21 - protein, 152 aa, synthetic construct
MNDYYTPVVSHRFMASFIFNGIPDPLDIRFQRISGLNRELQVTQHSQGGENARNNYLAEKIQHGTLTLERGVMTVSPLTWMFDRVLRGENIAYADVVIMLLNENSLPLSSWTLSNALPVRWQTSDFDANSNAILVNTLELRYQDMCWLGVKV

SEQ ID NO: 22 - protein, 65 aa, synthetic construct
MTVEIRELIIQAKVVSSSPILPTQATESHQQSHSLIQESLDEAALVEKIKREVLAALRDEEGWRP

SEQ ID NO: 23 - protein, 228 aa, synthetic construct
MSLIERGLAKLTINAYKDREGKIRAGTIQAMYNPDSLQLDYQTDYQQSQAINSEKQSSIYVQAKPAGLSLELIFDATMPGNKTPVEAQLMQLKQLCSVDATSNETRFLQIKWGKMRWENRGYFAGRAKGLSVNYTLFDRDATPLRARVILTLVADESLVLQETEQNLKSPAKIALRVQDGVSLALMAASTASTLSGGVDYLTLAWQNGLDNLNGFVPGEILQATRGDA

SEQ ID NO: 24 - protein, 538 aa, synthetic construct
MSHQLKIIADGKALSLLAAVDVDTYCRVNSIPSATLKLSLPDSPLSSFSQTDVQAELAHCQAGKTLRLELTDSGRKSVLFNGLITRNSLKIKNKQLLLTLVVRHRLQLMADTQHSQLFKASNEKTILNTLLNQAGIKARFERIDALDQKHEQMVQFRCSDWRFLLCRLSATGVWLLPTTEGAQLVQPNTLKSNPTHTLKSRGDEKKDIIVKDANWQFDNHLNPASLEVSGWDISKQQELSGGRHGSVAMGKAALSPDRLASLNKTSWDIRYSSPLTTQESGYLAQGLLLNQRISGVTGEFLLKGDGRYQLGDNIQLTGFGSQLDGTASITAVRHRFNRRIDWETTLSIGLPQEYLPMLPDATGLHIATVAKYQQDKAALNRIPIILPVLNRPNEFLWARLGKPYASHESGFCFYPEPGDEVIVGFFENDPRYPVILGAMHNPKNKAPLEPTQDNQEKVLVVKKGEIQQQIMINRKEKTIQMSAGENQIMLQQDKDISLSTKKELTLKAQTMNAEMEKSLNISGKNSVEIKGSKINLTQ

SEQ ID NO: 25 - protein, 140 aa, synthetic construct
MENQILTQLYGRGWAFPPVFSLEKGVEMAEGTEDVRQSLHILFSTEPGERLMRENYGCGLNDFMFENIRNELFAEIESHIHDSVLRYESRADITDIQVRQSPNSKNTLQVQVMYRLRGSDINQQIQGTLALGEGQGMEVV

SEQ ID NO: 26 - protein, 143 aa, synthetic construct
MSEPIVTDGDTLQFEPQFESRKVNIPGLIKINGTGHAQVNGKKVCILGDEKRVTVSATYTTTTHMTPGTGTITITALDSSQQALQCTSDAALIIKGKKFTAIFTPQSPAINGNVNPPQPDPNYPSPSSGKGSFITQQNFATVN

SEQ ID NO: 27 - protein, 736 aa, synthetic construct
MELTELNKKLSDLVPMSDFKLDSRTSLQLLQYIEEYTKIIPFNQTDKHWNDFFFKKDSTPEKLAELYQGKIEANGNLLPHQAFLLAVLRLLETPISLLNTLPAAHRNLYYRALLGLSPRPARPDQVALSVELNTTVTEQLLTKGTLFEAGQDEHGNALQYALDTSLLANRGYISELRWLRKKEQQQWITATPWNSQAQLSLPSGGIRLFSETDLDKSVLGGMLITSKHLAMEEGAREITITFDKDMDSQNLVAQIRSGNQWLTLQVEKNTAERNKKEVIMMLADKEPATRAPEDLDNLIFSEPVLRLQGKNSQPLPTVTALKVQKTTIDKASFKTFHLTPFGYSPEIEPLEENPALYLGITDVKPGQTLSLYWKLKSPQQPENVFWYYLNNKNQWVALDAWVKDETKYLYQDGIWQVVLPADASASAEEITRMPTGRYWLKAVMVIPTHKGSWGKTPWLDGLIYNAMTATLTNADSISNSHFLTPLPADTIQRPVEPIMEVASISQPWPSWNGRVPESYSAFFARGAQHLSHRNRALTWGNMATLLKERYVSIFDVKYPGHDELTRVPALEKQQLTIIPANQYNDSDDPLRPVLNPARLQGMAEWLQQKGSPWAEIEISNPQYIDVKINYNVIFKPDVNEDFGYRQLRQQLSETYMPWSVDEKRPVTLNNSISYYQLLATIQQQPLVERVTCLTLRRSEAAKDSDITASVEAKDNEVLILVWEADDKLQCRGNNYE

SEQ ID NO: 28 - protein, 963 aa, synthetic construct
MSNQDALFHSVKDDIHFDTLLEQAHQVVEQQAGKLWSDTAEHDPGITFLEGLSYGVSDLAYRHTLPPTDLLTPAPNEQKQQDGIFPAEFGPHNTLTCGPITTDDYRKALLDLHSSDWTGAKPESEQDKGDFLFRNVQLVREPETQRYTYWYDATKREYSFVERKDAKKFTLRGNYWLYLEPTRRTQENLDNATQQLIDFLTQNRNIGELVSQRIWTKPVDFPLLLDIELDDDVQNVAGIFAAVYSTAEQYLMPEAQRFSTETLQDAEMRNDEIFEGPRLEHGWIPELPTARDYTKRLKLNLSRLVNKLLEIKGIQNVNRLRLNENFDKTLIEPIKGDSWSWSIKEGYYPRLWGKDPIHQLAQHDGPLRVIAKGGISVTVDENSIRKSLSLSHPPLIQNKPVLLAYGRHRDVGRYYPVSDTLPACYKLQQPLSESEHAQRLLSLHQFMLPFEQLLACGCQQIAMLPKLLAFKREGYEVWGDQWPFKPGSVNDDAHQNYAYELKKVLKEIAHDNDHELDIVNYLLGYFGTQRAPRTFTTNISDFRAVQQGYLAQQPTLTYHRANIRIDQVSSLQKRIAARMGLGGELFKPKPDLSKLPFYLVEHRALLPVKPNSQFDEEQKPDSVTEERNYQNDQYYLVIKQAGIDGKLIQGQVIDLVLYEGEQNENRFTVRGQMITKTTGDQFWLDVSNSTQLEYNLERVMTAAKGKKLVWQNSPVWMEDMNYRLAYDSDQSSLPENQRRLTRTAQTPFPALIAAGNEITLTKQLGGVGLEQESSNESEKLYAKVVSFDRIKGTLIIERQKHSTLAFPAAEEAWRHSWHFSGKEYENTDRFSFVISVVVNSDLIKSRELKVDPYQLEEWVKETILTEFPAHISMIIHWMDREPFLNFGNTYQRWQNNGAPLGDAAYSILESLTLGKLPSAFKGIGSMRIATPHQREEVVGKNGEQWNTNRIKQNELFYIPKEKE

SEQ ID NO: 29 - protein, 419 aa, synthetic construct
MKEIRYSAKIQEQQTLSDAKGVGPDIDKLKDKFKEGSIPLQTDFNQLIDIADIGRKATGQAPNQNGPAKGMRLGEDGLLQLKLDEKYAHANYSPLRLHDDALVVGVGNGLINFKKSNEIGVNDGNGIRIDDNKVAVELADNKGLVVDSNGIAIKPGNGVKFSSDGALTVNSADSTIKVDGSGIKVATGWGVKVGGEGLDVNVRTDGGIGNDSSGIYVKTGNGIKLDNDQVAVELADNKGLVVDSNGIAIKPGDGMQFSSDGALQLKLNKNYADRFYSPLILRNDVLAVGISHGLTTYQGSYAIGVNPGNGLRINDDSVAVKLADNKGLVVDSNGISIKPGNGIKVDADGVAIDPNTVLPRGMIMMFSGNSVPEGWAICDGYNNTPDFLNRSIEGNTRNIKSKNGIDMTIQYTAIYIMKL

SEQ ID NO: 30 - protein, 511 aa, synthetic construct
MMTNTDKYGVNLINRITISIDMLYFNDDNIMENCSSIFNRKLKNIINKNIKNLTLNVNGKLSLERVTLDLGNIEIDLFEREITRRLEIELKKNLRNHYGYSQCILNKEKIYPHQSEKENRFLLIKEIDHYLHKGNWLSDHRKHHITNTVHINNELWQQINHQPQQWLPMLAKHCLQPAGLSRLIQLCQPDVLAMLCQLFTETTTSEFVNSQAQVITDKKVKPEKLSLAAEYYLQHQVKYPHATQQALAQQTQNKQTPTINIIQNNNSLLKQTYNETDMQMDTVLPFATYHQPTATQQHYGLIKEAVKQSLPTLQNREQHKELPRSTSPAKISSIQPSNGIQTPSSQSVLTISNAGCMILWPLLPIFFRTFDLLEKNQFISLEAQREAVCLLDWLIWEEEEIPAWRLTLNKILCGLPIHDNARWRTPKPEQQIAINQWLEKIIEQLPAWKKMGINDVRHLFLQRSGELSELNGIKNIHIKPEVYDALISEWAWPMNIASFSWLQHPITITWS

SEQ ID NO: 31 - protein, 695 aa, synthetic construct
MNTAPVFPDLFQQHNDPHLMFLYSQLERIDLVLQYHFHCISGQKGDLLDEFLLSEEDVINRLDNPLGKPHWLTDDCLTIPHTVTPVASRLTDLITHFELTDFERDVLLLGLLPHFDNRYYHLFALVQGEQQSRLPAFALALELFCHSMLEKQAQQASFLHQAPLVGCQLLSIDSRQKTLSWLQTPFITDSSVYHFLLGHHYIAPALEHCVEWITPTEIGNYPAGLKQALGNVLLSDHDDIRPVILLRGMADSARSHVVANMMASEQRQTLLVDIASLADNDDNSLFCHIKAILREIRMRGACLLLRNFCLFAEQNKHLLDPLSALLNQSELRVICLVEPHSPLVWLKKISTLLIEMPAFTSVEKARLLTAHLPNHCANDIDAITLSQRYAFNPETLPLILQEAKLYQQQRDPSGILQQCDIHKALNLRAQQNFGQLAQRITPKRSLKDLLVSDDIAQQIQEILAAIKYREHVLAGGFKDKIGYGTGISALFYGDSGTGKTMAAEVIANYIGVDLIKVDLSTVVNKYIGETEKNLSRIFDLAEQDAGVLFFDEADALFGKRSETKDAQDRHANIEVSYLLQRLENYPGLVILSTNNRSHLDNAFNRRFTFITRFTYPDETIRKKMWQAIWPENIKVAQDVDFDKLAQRTSVTGANIRNIALLSSLFAAENNHNEVSNKNIETALSRELAKVGRLIF

SEQ ID NO: 32 - protein, 301 aa, synthetic construct
MLKTQTIIDVNNAMKTMLEKYLDNKIAIRFDLPELDTVQSDAMVSVFLYDIHEDLQLRSTESRVFNATSGRLLPGWVNIKCNYLITYWESAQPATDSNSSECLPDNQAIKVMSQVLNALINNRQLAGIPGAYTQVVPPKESLNSLGNFWQSLGNRPRLSLNYSVTIPISLTDKQDKATPVSTISSTVEQIASLSQEKISHTLRELLITELQIQPVTESESEENIRLALSKVELLTMKKAITPDNSAEISISLSVSGITHQKYLQDINKIFDRWLNDNKIVTTVDNYGIRIKDIEKNHLFGI

SEQ ID NO: 33 - DNA, 309 bp, synthetic construct
  source 1..309: mol_type = other DNA
gtgtttatttcaaaagacttagcaaattttattgtcgtagccaaaaataaatcaataaataaggcaacaaaggagctttttattacacagtctccaattagccgaagcttaaaaaaattggagttctcattaggtgtaaaactctttgtcagaaaaaaccaaggattagttctaacggaagaaggggagtgtctatacaataaagtgttatcaatttatgaacaacttaaaaatatcgaaaatgattacaagaatcataaatcaccctattgtgaaatttataaaaaacaacataatgacttaacataa

SEQ ID NO: 34 - protein, 102 aa, synthetic construct
VFISKDLANFIVVAKNKSINKATKELFITQSPISRSLKKLEFSLGVKLFVRKNQGLVLTEEGECLYNKVLSIYEQLKNIENDYKNHKSPYCEIYKKQHNDLT

SEQ ID NO: 35 - DNA, 867 bp, synthetic construct
  source 1..867: mol_type = other DNA
gtgtatagtttaaaacagaaagaagagaagaaaaatcattcccctcgtcctacccaaaatactgtcaatggtgatcatgcaataacaccaagaatagcggaattgagaaaaaactttcagcagcttaattcgcaaaccgtgcgcccacgtgttgctcctcgtccattacattcactttcgaagacaggaccatttcaacaggctacaaaagcacctattgcctcagagataatcactcctgtcagcgcagctaccaaaacatttaccagtaatacacaaaacccaaaagtgacaccaacatcaacctctgcgccaacaaatggtgtaaaaaaatcatttacattatatcgagcagataaccgaagttttgaagagttacaaaaaagtagcccagagggatttaaggcttgggtacatcttgatagtgaaaaagcgagaaaatttgccagcgtattcttgggtaatgacaatgtagaaagtttacccaaacatattattgatgaaattaataaatggaaaaaaggaggaacacctaagttgagtgatctttccacatttataaaatataccaaagatcgctcaactgtttgggtttctaccgcagtcaatactgaagcaggtggacaaagctcaggagctccactttatgaaatatcaatggagctctatgaatttggggtagataaagggaaattggttccattacccaatggaagaacgggaaatatgaaaccttccattcatttggatacacaaaatctcgcagacgcaacaataatcgccctgaatcatgggccagttaatgatgctgaaatgtcatttttaacgactattccgatgagcaacttaaaaccctatagaaggtga

SEQ ID NO: 36 - DNA, 909 bp, synthetic construct
  source 1..909: mol_type = other DNA
atgatatacggttatgataacaagatggtttatagaaaaaggcaagaatcgaatacggcattggaagctttgcatcttgatatacccgatacagcggaagtctctgctgcctatcagcgcgatttgtcttctgtcatgacgagattccagaataaaacagactcaattcttgaggaatccaaacaaccctctccgctcaagcaaaaaccatcagagaaaaaaaaatatgctaaaaaggcattaaaaaactttgctgcccatgccggctactcacatatcaacagctatcaagatgagtttgttaactttaaagataacaattataacttagcccccggaaaattgttttggggtgtggaattaattccccaaaaaactatcgaaataaacagaccgataggaccatggagaaataaactttcctatgatatcgaagatatatttagaaataatatggcaaatgaatatcgggtaaccaatactttcgaatttatcaaaggattacaggatatgtataaaaaaaatgggcaaacgctacacccaatgacccaacaattggttgaagagcatattaaacataacgggaacatcttaccaacaatggcagggattgccggtttgcatgccgaagtacaggcattaaaccagttatttattaaagcagatgaggatgcaggccagtcccctgagccctttagtatgcgttatattaaggcaatgcttcaatcatcaattttcaccaaacgattgaccacagcgaacgccgggcaagacttcccggcttgccataactgctcgggtatcattcaatcaccagctaatgtgattacgggaacggtcagcagtgcaggcagcaatttttctaagcaggtcgcaaaacgcgatcgttcccagtcactaagtcaataa

SEQ ID NO: 37 - DNA, 1050 bp, synthetic construct
  source 1..1050: mol_type = other DNA
atgcccgtatatgaaaataaagaaaaaagaaagtattcaaaaaatcctttacataatacttcgactattaatcaatttactgttcaagatctggattctgcctcacagcaggaaacagcaacaccgctcctcaccaatgaatttaaacaaggccactatgtcaatcacagtaagttacctgctggtaccaaattatctgagatagccatgctgggtagccatgatgcgggaacttatgcttatagtaggagaaaatccggatttgccagtagcttagggtcactgcttcctgcggcatttaaaacccaaaatcgaacgttgaggcaacaagcagaagcaggagccagatatttcgatattcgggttgcgcaaaataaagatggctcatttagcttcttccatggccccagcgttgcaggcagtgatgccgtttcggatgtgaaatcgctcttggaatatgcggcaggagataccaatcacttttacttactcaaactcgtatttaaaggggaaaaagggcaatcttccgcagccgcgtcttcaaatacatttttacaaagtattctcgaaggccaccagcagcgtcttattacacttgatgatacgtcgagtttaggtgaggcgatggtcgatttactggataaaggaaaaaacatagggatcatggttgatagaaagaaatatgatggaacagaaccacattggggttataaagaaagtgttaacacaaagtgggctaacagagcgaacgcagaagaaacagcgaatttccttcttaaattccatgagaatccagtacctgacaaactcaatattatgcagaccaatatccctgttgcttccgtagggcgtgggcaatttacttcaggagtaaaaagatatttgtttggaaacagagacccattgatcaaagctgttgcccagcttcctgccggaataatcagcgcagattacgtaggcgattccggtagtgcaacttcaaaatttatggagacaattaatcaatataacaggagcttaatggaacgtgatgaagagaccagactgtaa

SEQ ID NO: 38 - protein, 288 aa, synthetic construct
VYSLKQKEEKKNHSPRPTQNTVNGDHAITPRIAELRKNFQQLNSQTVRPRVAPRPLHSLSKTGPFQQATKAPIASEIITPVSAATKTFTSNTQNPKVTPTSTSAPTNGVKKSFTLYRADNRSFEELQKSSPEGFKAWVHLDSEKARKFASVFLGNDNVESLPKHIIDEINKWKKGGTPKLSDLSTFIKYTKDRSTVWVSTAVNTEAGGQSSGAPLYEISMELYEFGVDKGKLVPLPNGRTGNMKPSIHLDTQNLADATIIALNHGPVNDAEMSFLTTIPMSNLKPYRR

SEQ ID NO: 39 - protein, 302 aa, synthetic construct
MIYGYDNKMVYRKRQESNTALEALHLDIPDTAEVSAAYQRDLSSVMTRFQNKTDSILEESKQPSPLKQKPSEKKKYAKKALKNFAAHAGYSHINSYQDEFVNFKDNNYNLAPGKLFWGVELIPQKTIEINRPIGPWRNKLSYDIEDIFRNNMANEYRVTNTFEFIKGLQDMYKKNGQTLHPMTQQLVEEHIKHNGNILPTMAGIAGLHAEVQALNQLFIKADEDAGQSPEPFSMRYIKAMLQSSIFTKRLTTANAGQDFPACHNCSGIIQSPANVITGTVSSAGSNFSKQVAKRDRSQSLSQ

SEQ ID NO: 40 - protein, 349 aa, synthetic construct
MPVYENKEKRKYSKNPLHNTSTINQFTVQDLDSASQQETATPLLTNEFKQGHYVNHSKLPAGTKLSEIAMLGSHDAGTYAYSRRKSGFASSLGSLLPAAFKTQNRTLRQQAEAGARYFDIRVAQNKDGSFSFFHGPSVAGSDAVSDVKSLLEYAAGDTNHFYLLKLVFKGEKGQSSAAASSNTFLQSILEGHQQRLITLDDTSSLGEAMVDLLDKGKNIGIMVDRKKYDGTEPHWGYKESVNTKWANRANAEETANFLLKFHENPVPDKLNIMQTNIPVASVGRGQFTSGVKRYLFGNRDPLIKAVAQLPAGIISADYVGDSGSATSKFMETINQYNRSLMERDEETRL

SEQ ID NO: 41 - DNA, 390 bp, synthetic construct
  source 1..390: mol_type = other DNA
gtgtatagtttaaaacagaaagaagagaagaaaaatcattcccctcgtcctacccaaaatactgtcaatggtgatcatgcaataacaccaagaatagcggaattgagaaaaaactttcagcagcttaattcgcaaaccgtgcgcccacgtgttgctcctcgtccattacattcactttcgaagacaggaccatttcaacaggctacaaaagcacctattgcctcagagataatcactcctgtcagcgcagctaccaaaacatttaccagtaatacacaaaacccaaaagtgacaccaacatcaacctctgcgccaacaaatggtgtaaaaaaatcatttacattatatcgagcagataaccgaagttttgaagagttacaaaaaagtagc

SEQ ID NO: 42 - DNA, 390 bp, synthetic construct
  source 1..390: mol_type = other DNA
atgatatacggttatgataacaagatggtttatagaaaaaggcaagaatcgaatacggcattggaagctttgcatcttgatatacccgatacagcggaagtctctgctgcctatcagcgcgatttgtcttctgtcatgacgagattccagaataaaacagactcaattcttgaggaatccaaacaaccctctccgctcaagcaaaaaccatcagagaaaaaaaaatatgctaaaaaggcattaaaaaactttgctgcccatgccggctactcacatatcaacagctatcaagatgagtttgttaactttaaagataacaattataacttagcccccggaaaattgttttggggtgtggaattaattccccaaaaaactatcgaaataaac

SEQ ID NO: 43 - DNA, 390 bp, synthetic construct
  source 1..390: mol_type = other DNA
atgcccgtatatgaaaataaagaaaaaagaaagtattcaaaaaatcctttacataatacttcgactattaatcaatttactgttcaagatctggattctgcctcacagcaggaaacagcaacaccgctcctcaccaatgaatttaaacaaggccactatgtcaatcacagtaagttacctgctggtaccaaattatctgagatagccatgctgggtagccatgatgcgggaacttatgcttatagtaggagaaaatccggatttgccagtagcttagggtcactgcttcctgcggcatttaaaacccaaaatcgaacgttgaggcaacaagcagaagcaggagccagatatttcgatattcgggttgcgcaaaataaagatggctcattt

SEQ ID NO: 44 - protein, 130 aa, synthetic construct
VYSLKQKEEKKNHSPRPTQNTVNGDHAITPRIAELRKNFQQLNSQTVRPRVAPRPLHSLSKTGPFQQATKAPIASEIITPVSAATKTFTSNTQNPKVTPTSTSAPTNGVKKSFTLYRADNRSFEELQKSS

SEQ ID NO: 45 - protein, 130 aa, synthetic construct
MIYGYDNKMVYRKRQESNTALEALHLDIPDTAEVSAAYQRDLSSVMTRFQNKTDSILEESKQPSPLKQKPSEKKKYAKKALKNFAAHAGYSHINSYQDEFVNFKDNNYNLAPGKLFWGVELIPQKTIEIN

SEQ ID NO: 46 - protein, 130 aa, synthetic construct
MPVYENKEKRKYSKNPLHNTSTINQFTVQDLDSASQQETATPLLTNEFKQGHYVNHSKLPAGTKLSEIAMLGSHDAGTYAYSRRKSGFASSLGSLLPAAFKTQNRTLRQQAEAGARYFDIRVAQNKDGSF

SEQ ID NO: 47 - DNA, 7714 bp, synthetic construct
  source 1..7714: mol_type = other DNA
attcctggattgcgccaaattatgtcttaagaaatttctataacccccaattatcacatctacacctccctattatttatctattaacaactttaacattcgatctttatttaatctttatttcactattaatattttacattttatctattaaatcatttttaacacgcattaattaaatgtcattaagcaattcttaaacaacttcttattttaagaaaaataaaattgcataaaaagcaatttgcattattggcaatgtactcattataaatttttcggcacgataaatatcgatataagcctgatacagccacatacaattttttcagagtgaagtttttttcagaatgaagtttactttcattttgtggcggtagctttatctgagcatatattttctgcatcctatttaatcaattacaaccatttttatttaaaaaagaggctactatgtctacaagcacatctcagattgctgttgaataccctattccttcttatcgtttcgttgtttccgtcggagatgaacatattccatttaatagtgtttcagggctggatattaattatgaaaccattgaataccgtgatggcgtgggtagttggtttaaaatgccgggtcagcgtcagccgattaatattaccctgcgtaaaggtgtttttccgggcaaaactgaattatttgactggattaattctatccaacttaatcaggttgagaaaaaagatatttccattagtttaaccaatgacgcaggcactgaattattaatgacctggaatgttgctaatgctttccctacctcattgacgtctccttcctttgatgccaccagcaatgatattgccgttcaggaaattaccctgacagccgatcgcgtcaccatgcaggctgtttgaggcattaatagttaatcatttcgtataaaggatttttttatgacaaccgttaccagttatcctggcgtttatattgaagaattaaatagcctggcattatccgtatcaaatagtgccaccgccgttcctgtttttgcagtgaacaaagaaaacaaacagattaatgaagagactgcacaccgaattaattcctggatggattatcttaatctggtaggcaactttgacaatgaggataaattgtcagtttctctgcgggcttattttaccaatggcgggggttattgttatctcatcaaaaccccaaatttagaaaaacttattccaaccttagatgatgtcactttgctggttgcggcaggtgaagatattaaaacagccgcggcaactttatgtcagccgggaaaagggttatttgccatttttgatggccctgaagaagcgttgaccatcgcgaatgcagaaacagtcaagaacaaatatgacgccaccgcgttcgccgcagtttactacccgtggctgaaaacggattgggcaaaaatcaccattccaccgagtgcggttatggcaggcgtttacgcctccgtcgatctctcccgtggcgtgtggaaagctcccgccaatatcgcattgaaaggcggactggaacctgcatttttgatcacggatgaagttcagagtgcatataactccggtcgtgccatcaatatgattcggaatttcagcaataccggtgccaccgtttggggagcaaggacgctggaagataatgacaactggcgctatgtccctgtgcgtcgcttattcaataccgtcgagcgggatgttaagcgcgctatgagctttgccatgtttgaacctaacagccaaccaacgtgggaacgtgtcagggcggcaatcagcaattaccttcatagcctgtggcaacaagggggattggctggcagcaaagaagaagatgcctatttcgtgcagattggcaaaggaattacgatgacgccagaccaaattaatcagggacaaatgatagtaaaaatcggcctggcggccgttcgaccggcagaatttatcatcctccagtttacgcaagatgtagaacagcgttaatcacattaattgatgaggaattatcatgccagctaatctaaaaacgcccggcgtttatattgaagaagatgcttcccttgcattatcggtcagcaacagtcccactgccgtgcctgtttttattggtaagttcaccccaaaaactgcggagccaacccaaacctgtattcgtatcagcaattggcttgaatttacttcctctttttctttggcaccagtgacagaaattgtcatccgctctagtcttgaagcctcttctgatggcgcaacaaaaaaagaacaggccaaaaaagaaaaagtcgaaaataaagagactgcaacccaagaaactcccaaagttcaaactctctcggcagccgaagaagaacccaaaaaatggattcacaatattgagagagtcaatctatctcaagccgtagaagccttgaagctctattttcaaaatggaggcggggcttgttatatctacccattaaacaatattaatggcgagtcggctctggaccccattcctaaggtgatagaacaaaaaggggatatcactctgttggtttgtccagaagaagatcagggttataaaaacagagtctacagtgcagtcagccccctattgaatagtgataacaaaaaagtgggctatttcctgattgcagatagccttgatggtaaatcggtgtctggcatggcaaatagcaccaagatcgccgcctattatcctcagttggaaacaaacctgaaattctccaccttgcccgacgatcagaacattgttatcagtggttatgagaacgcatcaggcaaggacaagctgaaaactctggataaacttagggaaacagataaagcgctggcacaagaaattgatatcagattgcaagaaatacaacaagataatctcaccctttcacccagtgctgccatcgcaggaatttattgccaaactgatagccagcgtggcgtctggaaagctcccgccaacgttgcactcagcggaatcaaaggtctgactgataaagtcgatgacgaacggcaaggcaccatgaatgagaatggcatcaatgtcatccgttcatttaccggccgtggcttgatggtttggggggcgcgtacttatgctcagaacggtgagatcaactggcgttacattcctgtccgtcgcctgttcaattccgttgaacgtgatatccgtcaggcactgcgtgccgtgttatttgaaaccaataatcaaccgacatggatgcgcgccaaggctgccgttgaccaatatctttatgccctctggcaaaaaaatgccctgatggggaacagcccggaagaggcttattttgtccatatcggtcaggatatcaccatgtctgatgcagatatcaaacaaggcaaaatgatcatgaaagtaggtctggccgcagtgcgaccggctgaatttatcgtcctgcaatttacgcaggatgtcgctcagtaatctccgtgattaaacaccgggcactgtattaacagtgcctatctcacccaattaaaggagatgatgatggaaagaattcaaccgggcgtgaccttgacagaaagtataattaccacaggccagcaagagatacccagcgcagtgccggtatttattggctataccgtccgcaatcaacaacaagcaaaaaccgcagttcgtatcgacaatctggcggaatatacccagcgatttggcgacgatcatctgatggcattggcggtaaggcactatttcgataatggcggacaacgggcttttgttttgccactgtcaggaaatatgccctcagcaaacatgacccaagcggaagccgaagcactgatggcggcattaagctctgacatggtgcaagaagccattggtggggaaacgcagatcaccctgattttggcaccggatatcgcccgactgaatgacaatgtgactgatgagcaacaaactttagtcaatttgtggtcacagggttggagtacactgctgcaactaagccagatccgcacgaatctctttgtgctgctggatgcgccggatgaggttgaacaggcacggcaatgtctggaaggactctcgtcagagtatcgccaatggggagccgcttattggcctcgtctggaaaccacttatcaggctacatccagttccaaaaatattatgctctcccccactgccgctatcgcagcacttatccaacacacggatagcgaagttggtgtatggaaagcgccagccaatattgccctgtctcaggttatccggccggttaagtcgtatcttcaagggagtgtactgtttgacaccaatggcacttcgctcaatgtgatccgcactttccccggcaaaggcatacgcgtatggggatgccgcacactggaaaacacagataacacgcagtggcgttacctacaaacacgacgtctggtttcttatgtcaccgtacatttggcgcaattagcccgtatgtacatctttgaacctaataacgaactgacgtggatgaaatgcaagggacaaagttacaactggctacggcaactgtggttacagggtggcttgtacggctcacgggaagatgaggcatttactgtgctgttaggcgtcaatgaaacgatgaccgaagaggatattcgtgccgggaaaatgataatgaaagtcgccttagccgtattgtctcccgcggaatttatcgagatcagtttggtatttgatacccaaacgggcgcgcttttgtcttaaaaaggaaagagcacaatgaacgattattacacccccgtggtatcccaccgttttatggcgagctttatttttaatggcattcctgatccactggatatccgttttcaacgtatttccggcctgaaccgggaacttcaggtcacccagcacagccaaggcggtgaaaacgcccgcaataactatctggctgaaaaaatccaacacggcacattaacgctggagcgcggtgtgatgacggtttctcctttgacctggatgtttgaccgtgtattgcgtggagaaaatatcgcctatgcggatgtggtgattatgctgttaaacgaaaattcgctgcccttgtccagttggacgctgagcaatgccttaccggtacgctggcagaccagcgattttgacgcgaacagtaatgccattctggtgaatacccttgaattgcgttatcaggatatgtgctggctgggagtcaaagtatgaccgtcgaaatcagagaattaattattcaggcaaaagtggtttcatcatcaccaatactcccaacacaagcaactgaatcacatcaacaaagccattctttgattcaggaaagtctggatgaggcagctttagttgaaaaaattaaacgcgaagtgctggctgcattacgcgatgaggaaggatggcgcccatgagtttaattgaacgtggtttagcgaagctgacgattaacgcttataaagacagggaaggaaaaatacgggctggcaccattcaggccatgtataaccctgattccctgcaactggattaccaaacggattaccaacaatcccaggcaattaatagcgaaaagcagagcagcatttatgtacaggccaagcctgccgggttatcccttgagctgatttttgacgccacaatgccgggcaacaaaacccctgttgaagctcagttaatgcagctcaagcagttgtgcagcgtggatgccaccagtaacgaaacgcggttcctgcaaatcaaatggggaaaaatgcgttgggaaaaccgcggctattttgctggcagggcgaaaggtttgtctgtgaattacaccttgtttgatcgtgatgccacgccattgcgggcgcgggtcatcctgacattggtggcggatgaaagtctggtcttacaggagacagagcaaaacctgaaatcgccggcgaaaattgccttacgggtacaggatggtgtttcgctggccctgatggcggcaagcaccgcatcaacgctgtctggtggtgttgattacctgacgctggcctggcaaaacggtctggataatcttaacggatttgtaccgggtgagatattgcaggccaccagaggagatgcctgatgagccatcaactgaaaatcattgccgatggcaaggcactgtctttgctggccgccgttgatgtcgatacttactgccgcgttaacagcatcccttccgcaacgctgaaactcagcctgccggacagccctctttcctctttcagccaaacggatgtacaggcagaactggcccattgtcaggcagggaaaaccctgcgtctggaattgactgacagcggcagaaaatcagtgctgtttaacggcctgattacccgtaactctttgaagataaaaaacaagcaattattgcttactttggttgtccgacatcggttgcaactgatggcagatactcagcactcacaactgtttaaggccagtaatgaaaaaaccattctgaacaccttattgaatcaggcgggtatcaaggctcgttttgagcggatagacgcactggatcaaaaacatgaacagatggtgcaatttcgctgttcagactggcgttttctgttgtgccgactatcggcaaccggcgtatggctgttacccacgacagaaggtgctcagcttgtccagcctaacaccctgaaatccaacccaacccataccctgaaaagccggggagatgagaaaaaagatatcatcgtcaaggatgccaactggcagtttgataaccatcttaaccctgcttcgctggaagtcagcggctgggatatcagtaaacagcaagaattatcaggtggtcgccacggcagtgttgccatgggcaaagccgcactttctcctgacaggctggcgtctttaaataaaacaagctgggacattcgctacagcagcccgttaaccacccaagagagtggctatctggcacagggactgttgttgaatcagcgcatttctggtgttacaggcgaattcctgcttaaaggtgatggacgttatcagttaggggacaacattcaattaacgggatttggttcacagctggatggaacagcaagcattactgcggttcgccatcgttttaaccggcgaattgattgggaaaccactttaagcattggcttaccacaggaatatctgccgatgctacccgatgccaccggactccatattgcgacagtcgcgaagtatcagcaggacaaggcagccctgaaccgcattccgattattctgccggtactgaatcgtccgaatgaattcttgtgggccagattagggaaaccttacgccagccacgaaagtggtttctgtttttacccagaacccggtgacgaagtgattgtcggcttttttgaaaatgatcctcgttatccggtgattctgggggcaatgcacaacccgaaaaataaagcgcctttagaacccacccaggataatcaggaaaaagtcttggtggtgaaaaaaggagaaatccaacaacaaatcatgattaatcgcaaagagaaaactattcaaatgagtgcaggagaaaaccagataatgctccagcaggataaagatatttcgctgtcaacgaaaaaagaattaacactgaaagcgcagaccatgaatgccgaaatggagaaatcactcaatatttctggcaaaaacagtgttgagatcaaaggcagcaaaattaatcttacccaatga

SEQ ID NO: 48 - DNA, 741 bp, synthetic construct
  source 1..741: mol_type = other DNA
gatgttagctttcgtctgagcggggcaaccagcagcagctatggtgtttttatttctaatctgcgtaaagcactgccgaatgaacgtaaactgtatgatattccgctgctgcgtagtagcctgccgggtagtcaacgttatgcactgattcatctgaccaattatgccgacgaaaccatcagcgtggcaattgacgttaccaatgtatatattatgggctatcgtgccggtgatacaagctatttttttaatgaagcaagcgcaaccgaagcagcaaaatatgtttttaaagacgccatgcgtaaagtgaccctgccgtatagtggtaactacgaacgcctgcaaacagcagcaggaaaaattcgtgaaaatatcccgctgggcctgccggcactggatagcgcaatcaccaccctgttttattataacgccaattctgcagcaagcgccctgatggttctgattcagagtacaagcgaagcagcacgttacaaatttattgaacagcagattgggaaacgtgtcgacaaaacctttctgccgtcactggcaattattagtctggaaaatagctggtctgcactgagcaaacaaatccaaattgcaagcaccaataacgggcagtttgaaagcccggttgttctgattaacgcccaaaatcagcgtgtgaccatcaccaatgtggacgcaggtgtcgttaccagcaacatcgccctgctgctgaatcgcaataatatggca

SEQ ID NO: 49 - DNA, 1108 bp, synthetic construct
  source 1..1108: mol_type = other DNA
ttagtcactcaagagtaatttgcctgcttttaacataatgatatcgcttatcagccaaacctagctctaataacatttaaattaatcttatgaataacaaggtttatttatcatattccatgaacattttattgttatttaataaggtttatttatttaaaaatcatattaattaatgtaataattcttatattcaattgttgacaaatattaatgtctatatatgattattgcacaattaataatttccactgtgatgaattaccacatcaaatcatgtaattaaaataaaaatgtaacaaatttattaataatttcataacaccaggaataagtcctattgaatttaaaaaggagtataggtgtttatttcaaaagacttagcaaattttattgtcgtagccaaaaataaatcaataaataaggcaacaaaggagctttttattacacagtctccaattagccgaagcttaaaaaaattggagttctcattaggtgtaaaactctttgtcagaaaaaaccaaggattagttctaacggaagaaggggagtgtctatacaataaagtgttatcaatttatgaacaacttaaaaatatcgaaaatgattacaagaatcataaatcaccctattgtgaaatttataaaaaacaacataatgacttaacataataaaataacaagatagataaaaatatatttcagataactattgaatcatattcaatagatttcattatatacataaattaaaaagtaaatttaacatgcctaaatatcttagagaagcagcagaagaaaagacttctgtacaaaaacattctaccgatagcaatcttctcaactcagggaactaatatcgcggatacctaacaatacaataatgcacttgaagaaagtgcattcaagttgaattaaaataaaacgttgaaggaaaagtatcacgaaccaccagctggacaggcagaaatccttttccccagcagagccaccttcaaggttcatgcgatcaagcgagatggcaaaaatacctatgtcttgctaagtgatatttcctctgatgccaacatagatacagatataaaagatatattttcaggaaaaaagat

SEQ ID NO: 50 - DNA, 861 bp, synthetic construct
  source 1..861: mol_type = other DNA
atgagtattcaacatttccgtgtcgcccttattcccttttttgcggcattttgccttcctgtttttgctcacccagaaacgctggtgaaagtaaaagatgctgaagatcagttgggtgcacgagtgggttacatcgaactggatctcaacagcggtaagatccttgagagttttcgccccgaagaacgtttcccaatgatgagcacttttaaagttctgctatgtggcgcggtattatcccgtgttgacgccgggcaagagcaactcggtcgccgcatacactattctcagaatgacttggttgagtactcaccagtcacagaaaagcatcttacggatggcatgacagtaagagaattatgcagtgctgccataaccatgagtgataacactgcggccaacttacttctgacaacgatcggaggaccgaaggagctaaccgcttttttgcacaacatgggggatcatgtaactcgccttgatcgttgggaaccggagctgaatgaagccataccaaacgacgagcgtgacaccacgatgcctgtagcaatggcaacaacgttgcgcaaactattaactggcgaactacttactctagcttcccggcaacaattaatagactggatggaggcggataaagttgcaggaccacttctgcgctcggcccttccggctggctggtttattgctgataaatctggagccggtgagcgtgggtctcgcggtatcattgcagcactggggccagatggtaagccctcccgtatcgtagttatctacacgacggggagtcaggcaactatggatgaacgaaatagacagatcgctgagataggtgcctcactgattaagcattggtaa

SEQ ID NO: 51 - DNA, 1032 bp, synthetic construct
  source 1..1032: mol_type = other DNA
atgtccaatttactgaccgtacaccaaaatttgcctgcattaccggtcgatgcaacgagtgatgaggttcgcaagaacctgatggacatgttcagggatcgccaggcgttttctgagcatacctggaaaatgcttcagtccgtttgccggtcgtgggcggcatggtgcaagttgaataaccggaaatggtttcccgcagaacctgaagatgttcgcgattatcttctatatcttcaggcgcgcggtctggcagtaaaaactatccagcaacatttgggccagctaaacatgcttcatcgtcggtccgggctgccacgaccaagtgacagcaatgctgtttcactggttatgcggcggatccgaaaagaaaacgttgatgccggtgaacgtgcaaaacaggctctagcgttcgaacgcactgatttcgaccaggttcgttcactcatggaaaatagcgatcgctgccaggatatacgtaatctggcatttctggggattgcttataacaccctgttacgtatagccgaaattgccaggatcagggttaaagatatctcacgtactgacggtgggagaatgttaatccatattggcagaacgaaaacgctggttagcaccgctggtgtagagaaggcacttagcctgggggtaactaaactggtcgagcgatggatttccgtctctggtgtagctgatgatccgaataactacctgttttgccgggtcagaaaaaatggtgttgccgcgccatctgccaccagccagctatcaactcgcgccctggaagggatttttgaagcaactcatcgattgatttacggcgctaaggatgactctggtcagagatacctggcctggtctggacacagtgcccgtgtcggagccgcgcgagatatggcccgcgctggagtttcaataccggagatcatgcaagctggtggctggaccaatgtaaatattgtcatgaactatatccgtaacctggatagtgaaacaggggcaatggtgcgcctgctggaagatggcgattaa

SEQ ID NO: 52 - DNA, 936 bp, synthetic construct
  source 1..936: mol_type = other DNA
atgaccagcaaagtttatgatccagaacagcgcaaacgtatgatcaccggcccgcagtggtgggcacgttgcaaacagatgaacgttctggatagctttatcaattattatgatagcgaaaaacatgccgaaaatgcagttatttttctgcatggtaatgccgccagttcatatctgtggcgtcatgttgttccacatattgaaccggtggcacgttgcatcattccggatctgattggtatgggtaaaagcggtaaaagcggcaatggtagttatcgtctgctggatcattataaatatctgaccgcgtggtttgaactgctgaatctgccgaaaaagatcatttttgttggtcatgattggggtgcatgtctggcatttcattatagctatgaacatcaggataaaatcaaagcaatcgttcatgcggaaagcgttgtagatgtcattgaaagttgggatgaatggccggatattgaagaagatattgcactgattaaaagcgaagaaggtgaaaaaatggttctggaaaataatttttttgttgaaaccatgctgccgagcaaaattatgcgtaaactggaaccggaagaatttgcagcatatctggaaccgtttaaagaaaaaggtgaagttcgtcgtccgaccctgagctggccgcgtgaaattccgctggttaaaggtggtaaaccggatgttgttcagattgttcgtaattataatgcatatctgcgtgcaagcgatgatctgccgaaaatgtttattgaaagcgatccgggtttttttagcaatgcaattgttgaaggtgcaaaaaaatttccgaataccgaatttgttaaagttaaaggtctgcattttagccaggaagatgcaccggatgaaatgggtaaatatattaaaagttttgttgaacgtgttctgaaaaatgaacagtaa

SEQ ID NO: 53 - DNA, 12139 bp, synthetic construct
  source 1..12139: mol_type = other DNA
aaggtgaacaatggaaaaccaaatactgacacagctttatggtcgtggctgggcttttcctcccgtcttttcccttgaaaagggggtggaaatggctgaggggacagaagatgtgcgccaaagtttgcatattctgttcagtactgagccgggggaacgcctgatgcgcgaaaattacggctgtggattaaatgattttatgtttgaaaatatccgcaacgaactgtttgctgaaattgaatcccatatccatgacagcgtattacgttatgaatcacgggcagatattaccgatatccaagttcgtcagtcgccaaatagcaaaaataccttgcaagtgcaggtgatgtatcgcctgcggggcagcgatatcaatcagcaaattcaaggaacactggcgctgggtgaaggccagggaatggaggtggtatgagtgaacccattgtaactgacggcgacacattacagtttgagccccaatttgagagtcgaaaggtgaacattcccggattgattaaaatcaatggaacaggtcatgcacaggtcaacggcaaaaaagtttgcattttgggagacgagaaacgggttactgtttctgcaacttataccacaacaactcatatgacaccgggaactggcaccattactatcacggcgttagatagcagccagcaagcccttcaatgtaccagtgatgctgctttaattatcaaagggaaaaaatttacggccatatttacgcctcaatcaccagccataaatggtaatgtgaatccacctcaacctgatcctaattacccaagcccttcatcaggcaaaggcagttttatcacccaacaaaactttgccactgtgaattaaggcattggctgaattaaatagaaattaaagggtgtgaataagtatttattcacagaggaatcgctgtgccacacaggtgatattatggaattaactgagttaaataaaaaattgtcagatttggtgccgatgagcgattttaaattagatagccgaaccagtttgcaattactccaatatattgaggagtacactaaaataattccctttaatcaaaccgataagcattggaatgattttttctttaagaaagatagtacgccagagaaactggccgaattatatcaagggaaaatcgaagccaatgggaatttattacctcatcaagcttttctactagcggtattacgattactggaaacaccaatatccttattgaataccttaccggcggcgcatcgcaatctctattatcgggcgcttttggggctatctccccgtccggctcgacctgatcaagttgccttatctgtagaactgaataccacagtcacagaacaactactcactaaaggcactttatttgaagcagggcaagatgaacacggcaatgccttgcaatatgcgctggataccagtttgctggcaaaccgtggctatattagtgaattgcgctggctccgtaaaaaagaacaacagcaatggatcaccgcgactccctggaattcacaggcacaattatcattgccatctggtggaatacggttattcagtgaaactgatttggataaatcggtactgggcgggatgttgatcacttccaaacatctggcgatggaagaaggagcaagagagataacgattacctttgataaggacatggatagccagaatttggtggcacaaatcagaagtggtaatcaatggctaactttacaagttgagaaaaatacagctgagagaaataaaaaagaagtcataatgatgctggcagataaagagccagcaacccgtgcaccagaggatctggataacctgattttcagtgagccagtactcaggctacagggaaaaaacagccaaccactgcctacagtcaccgcactaaaggtgcaaaaaacaactatagataaagcttcattcaagacatttcacttaaccccctttggttatagccctgaaattgaaccattggaagaaaaccccgcattataccttggtatcactgacgtcaagccgggacaaaccctatcgctgtattggaaattaaaatcgccacagcaacccgaaaacgttttctggtattacctgaataataagaatcaatgggttgcattagatgcgtgggtcaaagatgaaaccaaatatctgtatcaagatggcatctggcaagttgtattgcctgcggatgcttctgcttctgctgaagaaattacccggatgccaacagggcgctattggttaaaggcagtcatggttatccccacacacaaaggttcatggggaaaaactccttggttagacggcttgatctataacgccatgacagcgacattaacgaatgccgatagcatcagcaacagccatttcttgacgccattaccggcagacactattcaacgtcccgttgagcctatcatggaggtggcttcgatcagtcagccttggccgtcgtggaatgggcgtgtaccggaatcctacagcgctttttttgcacggggagctcaacatctgtcccaccgtaaccgcgccttaacctggggcaatatggcgacactgttaaaagagcgttatgtcagcatttttgatgttaagtaccccggccatgatgaactcacgcgagtccccgcactggagaaacagcaactgaccatcattccggctaaccaatacaacgacagcgatgatcctttgcgtccggtgttaaaccctgcccgcctgcaaggaatggccgaatggttacagcaaaaaggctctccatgggctgagattgagatcagcaatcctcaatacattgatgtaaaaatcaattacaacgtgatttttaagccggatgttaacgaagattttggttatcgccagctacgacagcaactcagcgagacatatatgccctggagcgtcgatgagaaacgccccgtcacgctgaataacagcattagttattaccaattactggcaactatccaacagcagccgctggttgagcgggtcacttgtctgacgctgcgtcggtcggaagcggctaaagacagtgatatcaccgcatcagtggaagccaaagataatgaagtgctgattttggtctgggaagcagatgacaagctgcaatgccgaggaaataactatgagtaatcaagatgcactatttcacagtgtgaaagacgatattcactttgataccttgctggaacaggctcatcaggtggttgagcaacaggcaggaaaattgtggagcgacacagcggaacacgatcccggtatcacctttctggaaggactcagttacggtgtgtcagatttagcttaccgtcatactcttcctccgacagacttactgacccctgcccctaatgagcagaaacagcaagatggaatttttcccgctgaatttggcccccacaatacactgacttgtgggccaatcaccactgatgattatcggaaggcattacttgatctgcatagcagtgactggacaggagcaaagccagagtcagaacaggacaaaggggattttctgttccgtaacgtgcaactggtacgtgaaccggaaacacaacgctatacctattggtatgatgccaccaaaagggaatatagctttgtcgagcgtaaagatgcgaaaaagtttaccctgcggggaaattattggctttatctggaaccgacccgtcgtactcaggagaatttggataatgctacccaacaattaatcgattttttgactcaaaaccgcaatattggtgaattggtcagtcagagaatctggacaaaaccggttgattttccgctattactggatattgaactggatgacgatgtgcaaaatgtcgctggtatttttgctgccgtctatagcacagcagaacagtatctgatgcctgaggcgcagcgtttcagtaccgaaacactacaagatgcggaaatgcgtaatgatgaaatctttgaaggaccacgattagaacatggctggatccctgaattgccgacagcccgtgattataccaaacggctcaagctcaatcttagccggctggtcaataagctgcttgagattaagggaatacagaatgtaaatcgtcttcgactgaatgaaaattttgataagaccctgattgagccgattaaaggggatagctggtcatggtcaataaaagaaggctactaccctcgtttgtggggtaaagatccgattcatcaattggcacaacatgatggcccactgagggtgatcgccaaaggtgggatcagcgttacggttgatgaaaacagcattcgaaaaagtttatccttatcccatcctcctcttattcagaataaacctgtgctattggcttatggtcggcatcgcgatgtgggtcgctattaccccgtcagcgatacgttgcccgcttgctacaaattacagcagcctttatctgaaagtgaacatgcgcaacgcctgttatcacttcatcaatttatgctgccatttgaacaattgttggcttgcggctgccagcaaattgccatgctgccaaaattgttggcttttaagcgtgagggatatgaagtttggggtgatcaatggccatttaagccgggttctgtcaatgatgatgcccaccaaaattacgcttacgaattaaagaaagtactaaaagagattgcacacgataacgatcacgaattggatattgtcaattatctgctcggatactttggcactcagcgagcaccacgtacctttaccaccaacatcagtgattttcgtgccgtgcaacaaggctatctggctcaacaaccgacattaacttatcaccgagccaatattcggatcgatcaagtttcgtcgctacaaaagcgcattgctgcccgtatggggttagggggtgaattatttaaaccaaagcctgacttgagcaaactgcctttttatctggtagaacatcgggcattgctgccagtcaaacccaacagccagtttgatgaagagcagaagccagattcggtgacagaagaaaggaactatcaaaatgatcaatattacttggtgattaagcaagccggtattgatggaaaactgatacagggacaggtaattgatttagttctctatgaaggagaacagaacgaaaaccgatttaccgtgcgtggtcaaatgatcactaaaaccacaggagatcagttttggctggacgtgagcaacagtactcaactggaatacaatctggaacgggtaatgaccgccgccaaagggaaaaaactcgtctggcaaaatagcccggtatggatggaagatatgaactaccggctggcctatgatagtgatcaatcctcattgcctgaaaaccagcggcgcctgacccgcacagcacaaacccccttcccggccctgattgccgcaggtaatgaaattaccctgacaaaacagttggggggagtgggtttggagcaagaatcttctaatgaatcagaaaaattatatgcaaaagttgtcagctttgatcgcatcaagggaactttgattattgagcgtcagaaacattctacactggcattccctgccgcagaagaagcctggcggcacagttggcatttttcgggtaaggaatatgaaaatacggaccgtttctcatttgtgattagcgtggtggtaaatagtgatttaattaaatcacgtgagctcaaagttgatccatatcaattggaagagtgggttaaggaaactattctcaccgaattccctgcccatatttccatgattattcactggatggatcgggagccatttttaaacttcggcaatacgtatcaacgttggcaaaataatggcgcaccattaggggatgccgcttattcgattctggaaagtttgacgctgggtaaattaccttccgctttcaaaggaattgggtcaatgcgtattgccacaccacatcagagagaggaagttgttggtaagaatggtgaacaatggaataccaatagaataaaacaaaacgaattattctatattccgaaagagaaagaataaaaaacaattagcgactaaccaacattttaaattaaaaatattttatggagttaacaatgaaagaaattcgttattctgcaaaaatacaagaacaacaaacattatctgacgcaaaaggtgttggacctgatattgataaattaaaagataagtttaaagaaggcagtattcccttacaaaccgatttcaatcaattaattgatattgccgatattgggcgtaaagcgactggacaggctcccaatcaaaatggcccggcaaaaggaatgcgtttgggcgaagatgggcttttacagttaaagttagatgagaaatacgctcatgcaaattacagtccattaagattgcatgatgatgcattggttgtaggagtaggcaatggtttgataaattttaaaaaatcaaatgaaataggtgttaatgatggaaatggtattaggatagatgataataaggttgcagtagaactggctgataataaaggtttggttgttgatagcaatggtatcgccataaaaccaggcaatggggtgaagtttagttcagatggtgcattaacagtaaattcggctgattcaactattaaagttgatggctcaggaataaaagttgctacaggttggggagttaaagttggtggtgaaggtttggatgtaaatgtccgcacggatggtggtattggtaatgattcgtcaggtatttatgttaaaacaggtaatggtattaagttagataatgatcaagttgcagtagaactagctgataataaaggtttagttgttgatagtaatggtatcgccataaaacccggcgatggaatgcaatttagttcagatggtgcattacagttaaaattaaataagaattatgccgatagattttatagccctttaatattgcgtaatgatgtattggctgtaggtataagccatggtttgacaacttatcaaggatcatatgcaataggtgttaatccaggaaatggtcttaggataaatgacgatagtgttgcagtgaaactagctgataataaaggcttggttgttgatagcaatggtatctccataaaaccaggcaatggaattaaggtagatgctgatggtgtggctatcgatcctaatactgtattgccacgtggtatgattatgatgttttctggtaatagcgtaccagaaggttgggctatttgtgatggctataataatacaccagattttctaaatagatctattgagggaaatactaggaatattaaaagtaaaaatggtatagatatgactatacaatatactgcaatatatatcatgaaattataattaacattaaacatggcaatgagcgttttaaaatacgctcattgaccaatttttggcaaggtggaatttgcgggttttatgatgaccaacactgataaatatggtgttaatcttattaatagaataactatctccattgatatgttatattttaacgatgataacataatggagaactgctcatctatatttaatagaaaactaaaaaatatcatcaataaaaatatcaaaaacctgacattgaatgtaaatgggaagttatctcttgaaagggtaactctggatctgggaaatattgaaattgatttatttgaaagggaaataacaagaagattggaaatagaattaaaaaagaacttaagaaatcattatggttactctcaatgtattttaaataaagagaaaatatatccacaccaatcagaaaaagaaaatagatttttattaataaaagaaatagatcattacttacataagggaaactggttatctgatcacagaaagcatcatattacaaatactgtgcatattaataatgaattatggcaacagattaaccaccagccacaacaatggctacctatgttagccaaacactgcttacagcctgcggggctaagtcgcttaattcaactctgccagccagacgttcttgctatgctttgccagttatttactgaaacaacaacatccgaatttgttaattcgcaagcgcaggtaattacagataaaaaagtgaaaccagaaaaattgagtttggctgcggaatattatctgcaacatcaggtgaaatatccccatgccacacaacaagcacttgcacaacaaactcaaaataagcaaacaccgacaataaatattattcagaataataacagtctattaaaacagacttacaatgaaactgatatgcagatggatacagtactgccatttgcaacataccatcagccaacagctacgcaacagcattatggtcttataaaagaggcggtaaaacaaagtcttccaactttacaaaacagagagcaacataaggaattaccgagatcaacttcaccagcgaaaatatcatccatacaacccagtaatggaattcagactccatcatcacaatccgttttaaccatcagcaatgccggttgcatgattttatggccgttattgcccatatttttccgtacctttgatttactggaaaagaatcaatttatcagccttgaagcacaaagagaggcggtctgtttacttgattggctgatttgggaagaagaggaaatacctgcatggcgattgactctcaataaaatactttgtggattacccatacatgacaacgcgcgatggcgtaccccaaagccagaacaacaaattgccatcaaccaatggctggaaaaaatcatcgaacaacttccagcctggaaaaaaatgggaataaacgatgtgcgacacttatttctgcaacgttccggggaattaagtgagttaaatggaataaaaaacatccatattaaacccgaagtttatgatgcactgataagcgaatgggcgtggccaatgaatatcgcgagctttagctggttgcaacaccctatcaccataacgtggtcataaccatcaaacacagtaaattagtctgagtaaaaatttatgaatacagcgcctgttttccctgatttatttcagcaacataatgatcctcatttaatgttcttatatagccaactggaacgcatcgatctcgttctgcaataccatttccattgcatatcaggccagaaaggtgacctccttgatgagttcttgttaagcgaagaagatgtgataaacagactggataaccctctgggaaaacctcattggctcaccgatgattgcctgacaataccgcacaccgtcacgcccgtggcatcccgattaactgacctgattacacattttgaactgactgattttgaaagggatgttttgttgttaggtttactgccccatttcgataaccgctactatcacctgtttgctctggttcagggagaacaacaatctcggctgcccgcttttgcgttggctttggaactgttttgccactcaatgctggaaaaacaggcacagcaggccagttttttacaccaggctcccttggttggctgccaactgttatctattgatagtcgtcagaaaacgttatcctggctccagacaccctttatcacagacagcagcgtatatcattttttacttgggcatcactatattgcacctgctctggaacattgtgttgagtggataacgcccacagaaatcggcaattatccagcaggattaaaacaagcgttgggtaatgtactgttatctgatcatgatgatatccggcccgttatcttactgcggggcatggccgatagtgccagatcccatgtcgttgctaatatgatggcatcagaacaacggcaaacgctgcttgtggatatcgccagcttagctgataacgatgacaactccctgttttgccatataaaagccattttgcgagaaattcgtatgcgtggtgcctgtttattgttacgaaacttttgcttatttgcagaacagaataaacacttgctggatcccctgtcagccttattaaaccaatctgaattaagggttatctgtctggttgaaccacactcaccgttagtatggctgaaaaagatatcgacattactgatcgaaatgcccgctttcacttcggtggaaaaagcaagattattgacggcccatttacccaatcactgtgcaaatgatatagatgcaataaccttaagccaacgttacgcatttaatcctgaaaccctgccattaattttacaagaggcgaaactttaccagcaacagcgagatccttcaggtattttgcagcaatgtgatatccataaggcactcaatttacgcgcccagcaaaattttggtcaattggcacaacgcattacccctaaacgttcattaaaagatttattggtatctgatgatattgctcaacagatacaagaaatactcgcagccattaagtatcgggaacacgtcctggcgggaggttttaaagataagattggttatggtacgggtatcagcgccctgttttatggtgattctggcaccggaaaaactatggcagcagaagtgattgccaattacattggcgttgacttaatcaaagtggatttatctaccgtcgtgaataaatacatcggcgaaacagagaaaaacttatcccgtatcttcgatttggcagaacaggatgccggtgttttattctttgatgaagcggatgcgttatttggtaaacgcagtgaaaccaaagatgcgcaagaccgacatgccaatattgaagtctcttatctactgcaacggctggagaactatccggggttggttattttatccaccaataatcgtagccatttggacaacgcctttaatcgccgttttacctttattacccgctttacttacccggatgaaaccatccgcaagaaaatgtggcaggcaatctggcctgaaaatataaaagtcgcccaggatgtggatttcgataaattagctcaacgaacaagcgtaacaggggcgaatattcgtaatattgctttattgtcttcactgtttgccgcagagaataaccataatgaagtcagtaataaaaatattgaaacagcattatcacgagaattagccaaagtaggccgtttaattttttaaaatttatagcaatgcaaatatctaacaattaaatgtactgataggttaattgttattaccattataaattaagaggattttttatgttaaaaacgcaaaccattattgatgtcaataacgcaatgaaaactatgctggagaaatatctggataataaaattgcaattcgttttgacttacctgaattagataccgtgcaatctgatgcgatggtgagtgtctttctgtatgatatccacgaagatctacagcttcgttcgacagaatccagagtgtttaatgccacttcagggagattattgccgggttgggtcaatattaaatgtaattacctgattacctattgggaatcggctcaaccagcaaccgattccaacagctcagaatgtctaccggataatcaggcaataaaagtcatgtcacaagtcttgaatgctctgattaataatcgccaattggcaggtattcccggtgcttatactcaggttgtccccccgaaagaaagtttaaacagtttagggaatttttggcaatcactggggaatcgcccccgactttctttaaattactcagtgacaataccgattagcctcaccgataagcaggataaggcgacgccggtaagcaccatttcttctacagtggaacaaattgcatcactcagtcaggaaaagattagccatactttgcgagaattattgattacggaactacagatacaacctgttacagaatcagaaagtgaagagaatatcaggctggcactgagcaaagttgaactattaacaatgaaaaaggctataactccagacaattcagcagaaatttccatatccttgtctgtatcaggtattacccatcagaaatatctacaggatatcaataaaatttttgatcgctggttaaatgacaacaaaattgttactacagtcgataattatggaatcaggattaaggatatagaaaaaaaccatcttttcggcatttaatttattgcttttccatagctcattaaataacagtttatttaaatcggagtattatt

SEQ ID NO: 54 - protein, 30 aa, synthetic construct
VYSLKQKEEKKNHSPRPTQNTVNGDHAITP

SEQ ID NO: 55 - protein, 30 aa, synthetic construct
MIYGYDNKMVYRKRQESNTALEALHLDIPD

SEQ ID NO: 56 - protein, 30 aa, synthetic construct
MPVYENKEKRKYSKNPLHNTSTINQFTVQD

SEQ ID NO: 57 - protein, 50 aa, synthetic construct
VYSLKQKEEKKNHSPRPTQNTVNGDHAITPRIAELRKNFQQLNSQTVRPR

SEQ ID NO: 58 - protein, 50 aa, synthetic construct
MIYGYDNKMVYRKRQESNTALEALHLDIPDTAEVSAAYQRDLSSVMTRFQ

SEQ ID NO: 59 - protein, 50 aa, synthetic construct
MPVYENKEKRKYSKNPLHNTSTINQFTVQDLDSASQQETATPLLTNEFKQ

SEQ ID NO: 60 - protein, 70 aa, synthetic construct
VYSLKQKEEKKNHSPRPTQNTVNGDHAITPRIAELRKNFQQLNSQTVRPRVAPRPLHSLSKTGPFQQATK

SEQ ID NO: 61 - protein, 70 aa, synthetic construct
MIYGYDNKMVYRKRQESNTALEALHLDIPDTAEVSAAYQRDLSSVMTRFQNKTDSILEESKQPSPLKQKP

SEQ ID NO: 62 - protein, 70 aa, synthetic construct
MPVYENKEKRKYSKNPLHNTSTINQFTVQDLDSASQQETATPLLTNEFKQGHYVNHSKLPAGTKLSEIAM

SEQ ID NO: 63 - protein, 90 aa, synthetic construct
VYSLKQKEEKKNHSPRPTQNTVNGDHAITPRIAELRKNFQQLNSQTVRPRVAPRPLHSLSKTGPFQQATKAPIASEIITPVSAATKTFTS

SEQ ID NO: 64 - protein, 90 aa, synthetic construct
MIYGYDNKMVYRKRQESNTALEALHLDIPDTAEVSAAYQRDLSSVMTRFQNKTDSILEESKQPSPLKQKPSEKKKYAKKALKNFAAHAGY

SEQ ID NO: 65 - protein, 90 aa, synthetic construct
MPVYENKEKRKYSKNPLHNTSTINQFTVQDLDSASQQETATPLLTNEFKQGHYVNHSKLPAGTKLSEIAMLGSHDAGTYAYSRRKSGFAS

SEQ ID NO: 66 - protein, 110 aa, synthetic construct
VYSLKQKEEKKNHSPRPTQNTVNGDHAITPRIAELRKNFQQLNSQTVRPRVAPRPLHSLSKTGPFQQATKAPIASEIITPVSAATKTFTSNTQNPKVTPTSTSAPTNGVK

SEQ ID NO: 67 - protein, 110 aa, synthetic construct
MIYGYDNKMVYRKRQESNTALEALHLDIPDTAEVSAAYQRDLSSVMTRFQNKTDSILEESKQPSPLKQKPSEKKKYAKKALKNFAAHAGYSHINSYQDEFVNFKDNNYNL

SEQ ID NO: 68 - protein, 110 aa, synthetic construct
MPVYENKEKRKYSKNPLHNTSTINQFTVQDLDSASQQETATPLLTNEFKQGHYVNHSKLPAGTKLSEIAMLGSHDAGTYAYSRRKSGFASSLGSLLPAAFKTQNRTLRQQ

SEQ ID NO: 69 - protein, 10 aa, synthetic construct
YCGTNYNGCY